European Patent Specification EP 3 619 325 B1, published January 24, 2024. Title: METHODS FOR TRAPPING AND BARCODING DISCRETE BIOLOGICAL UNITS IN HYDROGEL. Applicant: EDELSTEIN Stuart J. SCIPIO BIOSCIENCE. The sequence listing filed with the application follows.

SEQUENCE LISTING (2 sequences)

SEQ ID NO: 1 - DNA, 14 bp, Artificial Sequence
  Nucleic acid sequence primer
tcgtcggcagcgtc

SEQ ID NO: 2 - DNA, 14 bp, Artificial Sequence
  Nucleic acid sequence primer
gtctcgtgggctcg